European Patent Application EP 4 282 487 A2, published November 29, 2023. Title: FCRN ANTIBODIES AND METHODS OF USE THEREOF. Applicant: Momenta Pharmaceuticals, Inc. The sequence listing filed with the application follows.

SEQUENCE LISTING (62 sequences)

SEQ ID NO: 1 - protein, 14 aa, Homo sapiens
TGTGSDVGSYNLVS

SEQ ID NO: 2 - protein, 7 aa, Homo sapiens
GDSERPS

SEQ ID NO: 3 - protein, 10 aa, Homo sapiens
SSYAGSGIYV

SEQ ID NO: 4 - protein, 5 aa, Homo sapiens
TYAMG

SEQ ID NO: 5 - protein, 5 aa, Homo sapiens
DYAMG

SEQ ID NO: 6 - protein, 5 aa, Homo sapiens
NYAMG

SEQ ID NO: 7 - protein, 14 aa, Homo sapiens
SIGSSGAQTRYADS

SEQ ID NO: 8 - protein, 14 aa, Homo sapiens
SIGASGSQTRYADS

SEQ ID NO: 9 - protein, 14 aa, Homo sapiens
SIGASGAQTRYADS

SEQ ID NO: 10 - protein, 14 aa, Homo sapiens
SIGASGGQTRYADS

SEQ ID NO: 11 - protein, 7 aa, Homo sapiens
LAIGDSY

SEQ ID NO: 12 - protein, 14 aa, Homo sapiens
  SITE 1: note = MISC_FEATURE - Xaa is Gly, Leu, Ile, Ala, Phe, Met, Trp, Val, Pro, Ser, Thr, Cys, His, Tyr, Asn, or Gln
  SITE 12: note = MISC_FEATURE - Xaa is Gly, Leu, Ile, Ala, Phe, Met, Trp, Val, or Pro
XGTGSDVGSYNXVS

SEQ ID NO: 13 - protein, 7 aa, Homo sapiens
  SITE 3: note = MISC_FEATURE - Xaa is Ser, Thr, Cys, His, Met, Tyr, Trp, Asn, or Gln
  SITE 4: note = MISC_FEATURE - Xaa is Ser, Thr, Cys, His, Met, Tyr, Trp, Asn, Gln, Asp or Glu
GDXXRPS

SEQ ID NO: 14 - protein, 10 aa, Homo sapiens
  SITE 1: note = MISC_FEATURE - Xaa is Gly, Leu, Ile, Ala, Phe, Met, Trp, Val, Pro, Ser, Thr, Cys, His, Tyr, Asn, or Gln
  SITE 4: note = MISC_FEATURE - Xaa is Gly, Leu, Ile, Ala, Phe, Met, Trp, Val, or Pro
XSYXGSGIYV

SEQ ID NO: 15 - protein, 5 aa, Homo sapiens
  SITE 1: note = MISC_FEATURE - Xaa is Ser, Thr, Cys, His, Met, Tyr, Trp, Asn, Gln, Asp or Glu
XYAMG

SEQ ID NO: 16 - protein, 14 aa, Homo sapiens
  SITE 1: note = MISC_FEATURE - Xaa is Ser or Thr
  SITE 4: note = MISC_FEATURE - Xaa is Gly, Leu, Ile, Ala, Phe, Met, Trp, Val, Pro, Ser, Thr, Cys, His, Tyr, Asn, or Gln
  SITE 7: note = MISC_FEATURE - Xaa is Gly, Ser, or Ala
  SITE 10: note = MISC_FEATURE - Xaa is His, Lys, or Arg
XIGXSGXQTXYADS

SEQ ID NO: 17 - protein, 7 aa, Homo sapiens
  SITE 3: note = MISC_FEATURE - Xaa is Gly, Leu, Ile, Ala, Phe, Met, Trp, Val, Pro, His, Lys, or Arg
  SITE 4: note = MISC_FEATURE - Xaa is Gly, Ser, Asp, Gln, or His
LAXXDSY

SEQ ID NO: 18 - protein, 14 aa, Homo sapiens
  SITE 1: note = MISC_FEATURE - Xaa is Ser or Thr
  SITE 4: note = MISC_FEATURE - Xaa is Ser or Ala
  SITE 7: note = MISC_FEATURE - Xaa is Gly, Ser, or Ala
XIGXSGXQTRYADS

SEQ ID NO: 19 - protein, 216 aa, Homo sapiens
QSALTQPASVSGSPGQSITISCTGTGSDVGSYNLVSWYQQHPGKAPKLMIYGDSERPSGVSNRFSGSKSGNTASLTISGLQAEDEADYYCSSYAGSGIYVFGTGTKVTVLGQPKAAPSVTLFPPSSEELQANKATLVCLISDFYPGAVTVAWKADSSPVKAGVETTTPSKQSNNKYAASSYLSLTPEQWKSHKSYSCQVTHEGSTVEKTVAPTECS

SEQ ID NO: 20 - protein, 445 aa, Homo sapiens
EVQLLESGGGLVQPGGSLRLSCAASGFTFSTYAMGWVRQAPGKGLEWVSSIGSSGAQTRYADSVKGRFTISRDNSKNTLYLQMNSLRAEDTAVYYCARLAIGDSYWGQGTMVTVSSASTKGPSVFPLAPSSKSTSGGTAALGCLVKDYFPEPVTVSWNSGALTSGVHTFPAVLQSSGLYSLSSVVTVPSSSLGTQTYICNVNHKPSNTKVDKKVEPKSCDKTHTCPPCPAPELLGGPSVFLFPPKPKDTLMISRTPEVTCVVVDVSHEDPEVKFNWYVDGVEVHNAKTKPREEQYASTYRVVSVLTVLHQDWLNGKEYKCKVSNKALPAPIEKTISKAKGQPREPQVYTLPPSRDELTKNQVSLTCLVKGFYPSDIAVEWESNGQPENNYKTTPPVLDSDGSFFLYSKLTVDKSRWQQGNVFSCSVMHEALHNHYTQKSLSLSPG

SEQ ID NO: 21 - protein, 445 aa, Homo sapiens
EVQLLESGGGLVQPGGSLRLSCAASGFTFSDYAMGWVRQAPGKGLEWVSSIGASGSQTRYADSVKGRFTISRDNSKNTLYLQMNSLRAEDTAVYYCARLAIGDSYWGQGTMVTVSSASTKGPSVFPLAPSSKSTSGGTAALGCLVKDYFPEPVTVSWNSGALTSGVHTFPAVLQSSGLYSLSSVVTVPSSSLGTQTYICNVNHKPSNTKVDKKVEPKSCDKTHTCPPCPAPELLGGPSVFLFPPKPKDTLMISRTPEVTCVVVDVSHEDPEVKFNWYVDGVEVHNAKTKPREEQYASTYRVVSVLTVLHQDWLNGKEYKCKVSNKALPAPIEKTISKAKGQPREPQVYTLPPSRDELTKNQVSLTCLVKGFYPSDIAVEWESNGQPENNYKTTPPVLDSDGSFFLYSKLTVDKSRWQQGNVFSCSVMHEALHNHYTQKSLSLSPG

SEQ ID NO: 22 - protein, 445 aa, Homo sapiens
EVQLLESGGGLVQPGGSLRLSCAASGFTFSNYAMGWVRQAPGKGLEWVSSIGASGAQTRYADSVKGRFTISRDNSKNTLYLQMNSLRAEDTAVYYCARLAIGDSYWGQGTMVTVSSASTKGPSVFPLAPSSKSTSGGTAALGCLVKDYFPEPVTVSWNSGALTSGVHTFPAVLQSSGLYSLSSVVTVPSSSLGTQTYICNVNHKPSNTKVDKKVEPKSCDKTHTCPPCPAPELLGGPSVFLFPPKPKDTLMISRTPEVTCVVVDVSHEDPEVKFNWYVDGVEVHNAKTKPREEQYASTYRVVSVLTVLHQDWLNGKEYKCKVSNKALPAPIEKTISKAKGQPREPQVYTLPPSREEMTKNQVSLTCLVKGFYPSDIAVEWESNGQPENNYKTTPPVLDSDGSFFLYSKLTVDKSRWQQGNVFSCSVMHEALHNHYTQKSLSLSPG

SEQ ID NO: 23 - protein, 445 aa, Homo sapiens
EVQLLESGGGLVQPGGSLRLSCAASGFTFSTYAMGWVRQAPGKGLEWVSSIGASGGQTRYADSVKGRFTISRDNSKNTLYLQMNSLRAEDTAVYYCARLAIGDSYWGQGTMVTVSSASTKGPSVFPLAPSSKSTSGGTAALGCLVKDYFPEPVTVSWNSGALTSGVHTFPAVLQSSGLYSLSSVVTVPSSSLGTQTYICNVNHKPSNTKVDKKVEPKSCDKTHTCPPCPAPELLGGPSVFLFPPKPKDTLMISRTPEVTCVVVDVSHEDPEVKFNWYVDGVEVHNAKTKPREEQYASTYRVVSVLTVLHQDWLNGKEYKCKVSNKALPAPIEKTISKAKGQPREPQVYTLPPSREEMTKNQVSLTCLVKGFYPSDIAVEWESNGQPENNYKTTPPVLDSDGSFFLYSKLTVDKSRWQQGNVFSCSVMHEALHNHYTQKSLSLSPG

SEQ ID NO: 24 - protein, 445 aa, Homo sapiens
EVQLLESGGGLVQPGGSLRLSCAASGFTFSTYAMGWVRQAPGKGLEWVSSIGASGSQTRYADSVKGRFTISRDNSKNTLYLQMNSLRAEDTAVYYCARLAIGDSYWGQGTMVTVSSASTKGPSVFPLAPSSKSTSGGTAALGCLVKDYFPEPVTVSWNSGALTSGVHTFPAVLQSSGLYSLSSVVTVPSSSLGTQTYICNVNHKPSNTKVDKKVEPKSCDKTHTCPPCPAPELLGGPSVFLFPPKPKDTLMISRTPEVTCVVVDVSHEDPEVKFNWYVDGVEVHNAKTKPREEQYASTYRVVSVLTVLHQDWLNGKEYKCKVSNKALPAPIEKTISKAKGQPREPQVYTLPPSREEMTKNQVSLTCLVKGFYPSDIAVEWESNGQPENNYKTTPPVLDSDGSFFLYSKLTVDKSRWQQGNVFSCSVMHEALHNHYTQKSLSLSPG

SEQ ID NO: 25 - protein, 13 aa, Homo sapiens
KQGTWGGDWPEAL

SEQ ID NO: 26 - protein, 12 aa, Homo sapiens
FKALGGKGPYTL

SEQ ID NO: 27 - protein, 13 aa, Homo sapiens
GEEFMNFDLKQGT

SEQ ID NO: 28 - protein, 8 aa, Homo sapiens
EEFMNFDL

SEQ ID NO: 29 - protein, 9 aa, Homo sapiens
WGGDWPEAL

SEQ ID NO: 30 - protein, 280 aa, Homo sapiens
AESHLSLLYHLTAVSSPAPGTPAFWVSGWLGPQQYLSYNSLRGEAEPCGAWVWENQVSWYWEKETTDLRIKEKLFLEAFKALGGKGPYTLQGLLGCELGPDNTSVPTAKFALNGEEFMNFDLKQGTWGGDWPEALAISQRWQQQDKAANKELTFLLFSCPHRLREHLERGRGNLEWKEPPSMRLKARPSSPGFSVLTCSAFSFYPPELQLRFLRNGLAAGTGQGDFGPNSDGSFHASSSLTVKSGDEHHYCCIVQHAGLAQPLRVELESPAKSSHHHHHH

SEQ ID NO: 31 - protein, 99 aa, Homo sapiens [sequence omitted]

SEQ ID NO: 32 - protein, 220 aa, Homo sapiens
EVQLLESGGGLVQPGGSLRLSCAASGFTFSTYAMGWVRQAPGKGLEWVSSIGASGSQTRYADSVKGRFTISRDNSKNTLYLQMNSLRAEDTAVYYCARLAIGDSYWGQGTMVTVSSASTKGPSVFPLAPSSKSTSGGTAALGCLVKDYFPEPVTVSWNSGALTSGVHTFPAVLQSSGLYSLSSVVTVPSSSLGTQTYICNVNHKPSNTKVDKKVEPKSCD

SEQ ID NO: 33 - protein, 216 aa, Homo sapiens; identical to SEQ ID NO: 19

SEQ ID NO: 34 - protein, 6 aa, Homo sapiens
  SITE 3: note = MISC_FEATURE - Xaa is any amino acid
VGXYNL

SEQ ID NO: 35 - protein, 4 aa, Homo sapiens
GDSE

SEQ ID NO: 36 - protein, 7 aa, Homo sapiens
YAGSGIY

SEQ ID NO: 37 - skipped

SEQ ID NO: 38 - protein, 10 aa, Homo sapiens
SIGASGSQTR

SEQ ID NO: 39 - protein, 10 aa, Homo sapiens
  SITE 3: note = MISC_FEATURE - Xaa is any amino acid
  SITE 6: note = MISC_FEATURE - Xaa is any amino acid
  SITE 9: note = MISC_FEATURE - Xaa is any amino acid
SIXASXSQXR

SEQ ID NO: 40 - skipped

SEQ ID NO: 41 - protein, 14 aa, Homo sapiens
TIGSSGAQTRYADS

SEQ ID NO: 42 - protein, 14 aa, Homo sapiens
SIGASGSQTRYADS

SEQ ID NO: 43 - protein, 14 aa, Homo sapiens
TIGASGAQTRYADS

SEQ ID NO: 44 - protein, 14 aa, Homo sapiens
  SITE 4: note = MISC_FEATURE - Xaa is Ser or Ala
  SITE 7: note = MISC_FEATURE - Xaa is Gly, Ser, or Ala
SIGXSGXQTRYADS

SEQ ID NO: 45 - protein, 14 aa, Homo sapiens
  SITE 4: note = MISC_FEATURE - Xaa is Gly, Leu, Ile, Ala, Phe, Met, Trp, Val, Pro, Ser, Thr, Cys, His, Tyr, Asn, or Gln
  SITE 7: note = MISC_FEATURE - Xaa is Gly, Ser, or Ala
  SITE 10: note = MISC_FEATURE - Xaa is His, Lys, or Arg
SIGXSGXQTXYADS

SEQ ID NO: 46 - protein, 14 aa, Homo sapiens
TIGASGGQTRYADS

SEQ ID NO: 47 - protein, 8 aa, Homo sapiens
SDVGSYNL

SEQ ID NO: 48 - protein, 14 aa, Homo sapiens
  SITE 1: note = MISC_FEATURE - Xaa is Gly, Leu, Ile, Ala, Phe, Met, Trp, Val, Pro, Ser, Thr, Cys, His, Tyr, Asn, or Gln
XGTGSDVGSYNLVS

SEQ ID NO: 49 - protein, 14 aa, Homo sapiens
  SITE 12: note = MISC_FEATURE - Xaa is Gly, Leu, Ile, Ala, Phe, Met, Trp, Val, or Pro
TGTGSDVGSYNXVS

SEQ ID NO: 50 - protein, 7 aa, Homo sapiens
  SITE 3: note = MISC_FEATURE - Xaa is Ser, Thr, Cys, His, Met, Tyr, Trp, Asn, or Gln
GDXERPS

SEQ ID NO: 51 - protein, 7 aa, Homo sapiens
  SITE 4: note = MISC_FEATURE - Xaa is Ser, Thr, Cys, His, Met, Tyr, Trp, Asn, Gln, Asp or Glu
GDSXRPS

SEQ ID NO: 52 - protein, 10 aa, Homo sapiens
  SITE 1: note = MISC_FEATURE - Xaa is Gly, Leu, Ile, Ala, Phe, Met, Trp, Val, Pro, Ser, Thr, Cys, His, Tyr, Asn, or Gln
XSYAGSGIYV

SEQ ID NO: 53 - protein, 10 aa, Homo sapiens
  SITE 4: note = MISC_FEATURE - Xaa is Gly, Leu, Ile, Ala, Phe, Met, Trp, Val, or Pro
SSYXGSGIYV

SEQ ID NO: 54 - protein, 7 aa, Homo sapiens
  SITE 3: note = MISC_FEATURE - Xaa is Gly, Leu, Ile, Ala, Phe, Met, Trp, Val, Pro, His, Lys, or Arg
LAXGDSY

SEQ ID NO: 55 - protein, 7 aa, Homo sapiens
  SITE 4: note = MISC_FEATURE - Xaa is Gly, Ser, Asp, Gln, or His
LAIXDSY

SEQ ID NO: 56 - skipped

SEQ ID NO: 57 - protein, 6 aa, Homo sapiens
  SITE 3: note = MISC_FEATURE - Xaa is any amino acid
  SITE 6: note = MISC_FEATURE - Xaa is Gly, Leu, Ile, Ala, Phe, Met, Trp, Val, or Pro
VGXYNX

SEQ ID NO: 58 - skipped

SEQ ID NO: 59 - protein, 7 aa, Homo sapiens
  SITE 2: note = MISC_FEATURE - Xaa is Gly, Leu, Ile, Ala, Phe, Met, Trp, Val, or Pro
YXGSGIY

SEQ ID NO: 60 - skipped

SEQ ID NO: 61 - protein, 10 aa, Homo sapiens
  SITE 1: note = MISC_FEATURE - Xaa is Ser or Thr
  SITE 3: note = MISC_FEATURE - Xaa is any amino acid
  SITE 4: note = MISC_FEATURE - Xaa is Gly, Leu, Ile, Ala, Phe, Met, Trp, Val, Pro, Ser, Thr, Cys, His, Tyr, Asn, or Gln
  SITE 6: note = MISC_FEATURE - Xaa is any amino acid
  SITE 7: note = MISC_FEATURE - Xaa is Gly, Leu, Ile, Ala, Phe, Met, Trp, Val, Pro, His, Lys, or Arg
  SITE 9: note = MISC_FEATURE - Xaa is any amino acid
XIXXSXXQXR

SEQ ID NO: 62 - skipped